European Patent Application EP 4 151 082 A1, published March 22, 2023. Title: HIGH STEVIOL GLYCOSIDE-CONTENT STEVIA PLANT AND SCREENING METHOD THEREFOR. Applicant: SUNTORY HOLDINGS LIMITED. The sequence listing filed with the application follows.

SEQUENCE LISTING (37 sequences)

SEQ ID NO: 1 - DNA, 326 bp, Stevia rebaudiana
ggcagccattgatgatgttgttgaatgtgattaatttgaatgttataaagaatttggaaaagaaaaaggaggggacaaagttgatgaaattaggggagttatgattatgatggccatggtgattgtgatgagtggcactatgtaatctaatatttgaagatatgagaccacttgaccatgttataatcttatacaaaataattaatccctcacggtaatttttttctaatccttaaactgaaatttgaaagtaatttgagatagtgtttcccctaatttatgcttttagtatgcatttattctatcatattttctatgagaattgg

SEQ ID NO: 2 - DNA, 145 bp, Stevia rebaudiana
gatccaatggagggggtgattcaggtaataaaaggcattagtatggaatataccaaaacattgcgattcgttattagcatggatctttcaagtaataaacttatcggagaaataccagttgagttaactgcccttcatgccttgg

SEQ ID NO: 3 - DNA, 25 bp, Artificial Sequence
  Synthetic DNA
ggcagccattgatgatgttgttgaa

SEQ ID NO: 4 - DNA, 36 bp, Artificial Sequence
  Synthetic DNA
ccaattctcatagaaaatatgatagaataaatgcat

SEQ ID NO: 5 - DNA, 21 bp, Artificial Sequence
  Synthetic DNA
gatccaatggagggggtgatt

SEQ ID NO: 6 - DNA, 21 bp, Artificial Sequence
  Synthetic DNA
ccaaggcatgaagggcagtta

SEQ ID NO: 7 - DNA, 21 bp, Stevia rebaudiana
atgcttttagtatgcatttat

SEQ ID NO: 8 - DNA, 41 bp, Stevia rebaudiana
cccctaatttatgcttttagtatgcatttattctatcatat

SEQ ID NO: 9 - DNA, 61 bp, Stevia rebaudiana
gatagtgtttcccctaatttatgcttttagtatgcatttattctatcatattttctatgag

SEQ ID NO: 10 - DNA, 21 bp, Stevia rebaudiana
aaaaggcattagtatggaata

SEQ ID NO: 11 - DNA, 41 bp, Stevia rebaudiana
ttcaggtaataaaaggcattagtatggaatataccaaaaca

SEQ ID NO: 12 - DNA, 61 bp, Stevia rebaudiana
gagggggtgattcaggtaataaaaggcattagtatggaatataccaaaacattgcgattcg

SEQ ID NO: 13 - DNA, 326 bp, Stevia rebaudiana
ggcagccattgatgatgttgttgaatgtgattaatttgaatgttataaagaatttggaaaagaaaaaggaggggacaaagttgatgaaattaggggagttatgattatgatggccatggtgattgtgatgagtggcactatgtaatctaatatttgaagatatgagaccacttgaccatgttataatcttatacaaaataattaatccctcacggtaatttttttctaatccttaaactgaaatttgaaagtaatttgagatagtgtttcccctaatttatgcttttagcatgcatttattctatcatattttctatgagaattgg

SEQ ID NO: 14 - DNA, 21 bp, Stevia rebaudiana
atgcttttagcatgcatttat

SEQ ID NO: 15 - DNA, 41 bp, Stevia rebaudiana
cccctaatttatgcttttagcatgcatttattctatcatat

SEQ ID NO: 16 - DNA, 61 bp, Stevia rebaudiana
gatagtgtttcccctaatttatgcttttagcatgcatttattctatcatattttctatgag

SEQ ID NO: 17 - DNA, 145 bp, Stevia rebaudiana
gatccaatggagggggtgattcaggtaataaaaggcattcgtatggaatataccaaaacattgcgattcgttattagcatggatctttcaagtaataaacttatcggagaaataccagttgagttaactgcccttcatgccttgg

SEQ ID NO: 18 - DNA, 21 bp, Stevia rebaudiana
aaaaggcattcgtatggaata

SEQ ID NO: 19 - DNA, 41 bp, Stevia rebaudiana
ttcaggtaataaaaggcattcgtatggaatataccaaaaca

SEQ ID NO: 20 - DNA, 61 bp, Stevia rebaudiana
gagggggtgattcaggtaataaaaggcattcgtatggaatataccaaaacattgcgattcg

SEQ ID NO: 21 - DNA, 25 bp, Artificial Sequence
  Synthetic DNA
ggcagccattgatgatgttgttgaa

SEQ ID NO: 22 - DNA, 36 bp, Artificial Sequence
  Synthetic DNA
ccaattctcatagaaaatatgatagaataaatgcgt

SEQ ID NO: 23 - DNA, 36 bp, Artificial Sequence
  Synthetic DNA
ccaattctcatagaaaatatgatagaataaatgtat

SEQ ID NO: 24 - DNA, 36 bp, Artificial Sequence
  Synthetic DNA
ccaattctcatagaaaatatgatagaataaatgcaa

SEQ ID NO: 25 - DNA, 48 bp, Artificial Sequence
  Synthetic DNA
ttatttaatgatccaatggagggggtgattcaggtaataaaaggcact

SEQ ID NO: 26 - DNA, 48 bp, Artificial Sequence
  Synthetic DNA
ttatttaatgatccaatggagggggtgattcaggtaataaaaggctta

SEQ ID NO: 27 - DNA, 48 bp, Artificial Sequence
  Synthetic DNA
ttatttaatgatccaatggagggggtgattcaggtaataaaagtcatg

SEQ ID NO: 28 - DNA, 28 bp, Artificial Sequence
  Synthetic DNA
tgagggttctcaattgatttccgattgg

SEQ ID NO: 29 - DNA, 367 bp, Stevia rebaudiana
ttatttaatgatccaatggagggggtgattcaggtaataaaaggcattagtatggaatataccaaaacattgcgattcgttattagcatggatctttcaagtaataaacttatcggagaaataccagttgagttaactgcccttcatgccttggtgagtctcaatttgtctaataatcatcttattggacacattccgaatagcattggaaacatgaaagctttaaattctctagatttctcgagaaacgagttaaatgggttgatccctccaagcattggagctttgaattttttgagtcatttaaatttgtcaaacaacaacttatcaggaccaattccaatcggaaatcaattgagaaccctca

SEQ ID NO: 30 - DNA, 326 bp, Artificial Sequence
  Synthetic DNA
ggcagccattgatgatgttgttgaatgtgattaatttgaatgttataaagaatttggaaaagaaaaaggaggggacaaagttgatgaaattaggggagttatgattatgatggccatggtgattgtgatgagtggcactatgtaatctaatatttgaagatatgagaccacttgaccatgttataatcttatacaaaataattaatccctcacggtaatttttttctaatccttaaactgaaatttgaaagtaatttgagatagtgtttcccctaatttatgcttttagtacgcatttattctatcatattttctatgagaattgg

SEQ ID NO: 31 - DNA, 290 bp, Artificial Sequence
  Synthetic DNA
ggcagccattgatgatgttgttgaatgtgattaatttgaatgttataaagaatttggaaaagaaaaaggaggggacaaagttgatgaaattaggggagttatgattatgatggccatggtgattgtgatgagtggcactatgtaatctaatatttgaagatatgagaccacttgaccatgttataatcttatacaaaataattaatccctcacggtaatttttttctaatccttaaactgaaatttgaaagtaatttgagatagtgtttcccctaatttatgcttttagt

SEQ ID NO: 32 - DNA, 36 bp, Artificial Sequence
  Synthetic DNA
acgcatttattctatcatattttctatgagaattgg

SEQ ID NO: 33 - DNA, 326 bp, Artificial Sequence
  Synthetic DNA
ggcagccattgatgatgttgttgaatgtgattaatttgaatgttataaagaatttggaaaagaaaaaggaggggacaaagttgatgaaattaggggagttatgattatgatggccatggtgattgtgatgagtggcactatgtaatctaatatttgaagatatgagaccacttgaccatgttataatcttatacaaaataattaatccctcacggtaatttttttctaatccttaaactgaaatttgaaagtaatttgagatagtgtttcccctaatttatgcttttagcacgcatttattctatcatattttctatgagaattgg

SEQ ID NO: 34 - DNA, 367 bp, Artificial Sequence
  Synthetic DNA
ttatttaatgatccaatggagggggtgattcaggtaataaaaggcactagtatggaatataccaaaacattgcgattcgttattagcatggatctttcaagtaataaacttatcggagaaataccagttgagttaactgcccttcatgccttggtgagtctcaatttgtctaataatcatcttattggacacattccgaatagcattggaaacatgaaagctttaaattctctagatttctcgagaaacgagttaaatgggttgatccctccaagcattggagctttgaattttttgagtcatttaaatttgtcaaacaacaacttatcaggaccaattccaatcggaaatcaattgagaaccctca

SEQ ID NO: 35 - DNA, 367 bp, Artificial Sequence
  Synthetic DNA
ttatttaatgatccaatggagggggtgattcaggtaataaaaggcactcgtatggaatataccaaaacattgcgattcgttattagcatggatctttcaagtaataaacttatcggagaaataccagttgagttaactgcccttcatgccttggtgagtctcaatttgtctaataatcatcttattggacacattccgaatagcattggaaacatgaaagctttaaattctctagatttctcgagaaacgagttaaatgggttgatccctccaagcattggagctttgaattttttgagtcatttaaatttgtcaaacaacaacttatcaggaccaattccaatcggaaatcaattgagaaccctca

SEQ ID NO: 36 - DNA, 46 bp, Artificial Sequence
  Synthetic DNA
ttatttaatgatccaatggagggggtgattcaggtaataaaaggca

SEQ ID NO: 37 - DNA, 320 bp, Artificial Sequence
  Synthetic DNA
ctagtatggaatataccaaaacattgcgattcgttattagcatggatctttcaagtaataaacttatcggagaaataccagttgagttaactgcccttcatgccttggtgagtctcaatttgtctaataatcatcttattggacacattccgaatagcattggaaacatgaaagctttaaattctctagatttctcgagaaacgagttaaatgggttgatccctccaagcattggagctttgaattttttgagtcatttaaatttgtcaaacaacaacttatcaggaccaattccaatcggaaatcaattgagaaccctc